European Patent Application EP 4 328 243 A1, published February 28, 2024. Title: Asymmetric antibody with enhanced target cell clearance. Applicant: SG Medical, Inc. The sequence listing filed with the application follows.

SEQUENCE LISTING (54 sequences)

SEQ ID NO: 1 - DNA, 41 bp, Artificial Sequence
  VL Primer (F) CD20-scFv-knob
cgcagcgagcgcgcactcccagatcgtcctgagtcagagcc

SEQ ID NO: 2 - DNA, 86 bp, Artificial Sequence
  VL Primer (R) CD20-scFv-knob
agagccgccagatccactgcctcctccaccgctaccgccaccaccactcccgcctccgcccttaatctccaatttagttcccccgc

SEQ ID NO: 3 - DNA, 41 bp, Artificial Sequence
  VH Primer (F) CD20-scFv-knob
gcagtggatctggcggctctcaggtccagctccaacagccc

SEQ ID NO: 4 - DNA, 55 bp, Artificial Sequence
  VH Primer (R) CD20-scFv-knob
ggtgggcatgtgtgagttttgtctgagccgccagcactcaccgtcacagtggtac

SEQ ID NO: 5 - DNA, 23 bp, Artificial Sequence
  CH Primer (F) CD20-scFv-knob
gacaaaactcacacatgcccacc

SEQ ID NO: 6 - DNA, 33 bp, Artificial Sequence
  CH Primer (R) CD20-scFv-knob
ctctccctgtccccgggtaaatgactagaacta

SEQ ID NO: 7 - DNA, 45 bp, Artificial Sequence
  VL- CK Primer (F) CD20-Fab-hole
cgcagcgagcgcgcactcccagattgtcctgtctcagtctcctgc

SEQ ID NO: 8 - DNA, 44 bp, Artificial Sequence
  VL- CK Primer (R) CD20-Fab-hole
cggccgccgtgcgagatcttttgatttccagtttagttccgccg

SEQ ID NO: 9 - DNA, 23 bp, Artificial Sequence
  VH Primer (F) CD20-Fab-hole
caagtccaactgcaacaaccggg

SEQ ID NO: 10 - DNA, 50 bp, Artificial Sequence
  VH Primer (R) CD20-Fab-hole
ggaagaccgatgggcccttgaagctagcggcggaaaccgttgtgccagag

SEQ ID NO: 11 - DNA, 15 bp, Artificial Sequence
  CH Primer (F) CD20-Fab-hole
gcaagcttcaagggc

SEQ ID NO: 12 - DNA, 33 bp, Artificial Sequence; identical to SEQ ID NO: 6
  CH Primer (R) CD20-Fab-hole

SEQ ID NO: 13 - protein, 477 aa, Artificial Sequence
  CD20-scFv-knob
QIVLSQSPAILSASPGEKVTMTCRASSSVSYIHWFQQKPGSSPKPWIYATSNLASGVPVRFSGSGSGTSYSLTISRVEAEDAATYYCQQWTSNPPTFGGGTKLEIKGGGGSGGGGSGGGGSGSGGSQVQLQQPGAELVKPGASVKMSCKASGYTFTSYNMHWVKQTPGRGLEWIGAIYPGNGDTSYNQKFKGKATLTADKSSSTAYMQLSSLTSEDSAVYYCARSTYYGGDWYFNVWGAGTTVTVSAGGSDKTHTCPPCPAPELLGGPSVFLFPPKPKDTLMISRTPEVTCVVVDVSHEDPEVKFNWYVDGVEVHNAKTKPREEQYNSTYRVVSVLTVLHQDWLNGKEYKCKVSNKALPAPIEKTISKAKGQPREPQVYTLPPSRDELTKNQVSLWCLVKGFYPSDIAVEWESNGQPENNYKTTPPVLDSDGSFFLYSKLTVDKSRWQQGNVFSCSVMHEALHNHYTQKSLSLSPGK

SEQ ID NO: 14 - protein, 706 aa, Artificial Sequence
  CD20-Fab-hole
QIVLSQSPAILSASPGEKVTMTCRASSSVSYIHWFQQKPGSSPKPWIYATSNLASGVPVRFSGSGSGTSYSLTISRVEAEDAATYYCQQWTSNPPTFGGGTKLEIKRSRTAAAPSVFIFPPSDEQLKSGTASVVCLLNNFYPREAKVQWKVDNALQSGNSQESVTEQDSKDSTYSLSSTLTLSKADYEKHKVYACEVTHQGLSSPVTKSFNRGECGGGGSGGGGSGGGGSGSGGSGGGGSGGGGSGGGGSGSGSSQVQLQQPGAELVKPGASVKMSCKASGYTFTSYNMHWVKQTPGRGLEWIGAIYPGNGDTSYNQKFKGKATLTADKSSSTAYMQLSSLTSEDSAVYYCARSTYYGGDWYFNVWGAGTTVTVSAASFKGPSVFPLAPSSKSTSGGTAALGCLVKDYFPEPVTVSWNSGALTSGVHTFPAVLQSSGLYSLSSVVTVPSSSLGTQTYICNVNHKPSNTKVDKKVEPKSCDKTHTCPPCPAPELLGGPSVFLFPPKPKDTLMISRTPEVTCVVVDVSHEDPEVKFNWYVDGVEVHNAKTKPREEQYNSTYRVVSVLTVLHQDWLNGKEYKCKVSNKALPAPIEKTISKAKGQPREPQVYTLPPSRDELTKNQVSLSCAVKGFYPSDIAVEWESNGQPENNYKTTPPVLDSDGSFFLVSKLTVDKSRWQQGNVFSCSVMHEALHNHYTQKSLSLSPGK

SEQ ID NO: 15 - protein, 23 aa, Artificial Sequence
  LFR1 of CD20-scFv-knob
QIVLSQSPAILSASPGEKVTMTC

SEQ ID NO: 16 - protein, 10 aa, Artificial Sequence
  LCDR1 of CD20-scFv-knob
RASSSVSYIH

SEQ ID NO: 17 - protein, 15 aa, Artificial Sequence
  LFR2 of CD20-scFv-knob
WFQQKPGSSPKPWIY

SEQ ID NO: 18 - protein, 7 aa, Artificial Sequence
  LCDR2 of CD20-scFv-knob
ATSNLAS

SEQ ID NO: 19 - protein, 32 aa, Artificial Sequence
  LFR3 of CD20-scFv-knob
GVPVRFSGSGSGTSYSLTISRVEAEDAATYYC

SEQ ID NO: 20 - protein, 9 aa, Artificial Sequence
  LCDR3 of CD20-scFv-knob
QQWTSNPPT

SEQ ID NO: 21 - protein, 10 aa, Artificial Sequence
  LFR4 of CD20-scFv-knob
FGGGTKLEIK

SEQ ID NO: 22 - protein, 20 aa, Artificial Sequence
  Linker of CD20-scFv-knob
GGGGSGGGGSGGGGSGSGGS

SEQ ID NO: 23 - protein, 30 aa, Artificial Sequence
  HFR1 of CD20-scFv-knob
QVQLQQPGAELVKPGASVKMSCKASGYTFT

SEQ ID NO: 24 - protein, 5 aa, Artificial Sequence
  HCDR1 of CD20-scFv-knob
SYNMH

SEQ ID NO: 25 - protein, 14 aa, Artificial Sequence
  HFR2 of CD20-scFv-knob
WVKQTPGRGLEWIG

SEQ ID NO: 26 - protein, 17 aa, Artificial Sequence
  HCDR2 of CD20-scFv-knob
AIYPGNGDTSYNQKFKG

SEQ ID NO: 27 - protein, 32 aa, Artificial Sequence
  HFR3 of CD20-scFv-knob
KATLTADKSSSTAYMQLSSLTSEDSAVYYCAR

SEQ ID NO: 28 - protein, 12 aa, Artificial Sequence
  HCDR3 of CD20-scFv-knob
STYYGGDWYFNV

SEQ ID NO: 29 - protein, 11 aa, Artificial Sequence
  HFR4 of CD20-scFv-knob
WGAGTTVTVSA

SEQ ID NO: 30 - protein, 120 aa, Artificial Sequence
  CH2 of CD20-scFv-knob
DKTHTCPPCPAPELLGGPSVFLFPPKPKDTLMISRTPEVTCVVVDVSHEDPEVKFNWYVDGVEVHNAKTKPREEQYNSTYRVVSVLTVLHQDWLNGKEYKCKVSNKALPAPIEKTISKAK

SEQ ID NO: 31 - protein, 107 aa, Artificial Sequence
  CH3 of CD20-scFv-knob
GQPREPQVYTLPPSRDELTKNQVSLWCLVKGFYPSDIAVEWESNGQPENNYKTTPPVLDSDGSFFLYSKLTVDKSRWQQGNVFSCSVMHEALHNHYTQKSLSLSPGK

SEQ ID NO: 32 - protein, 23 aa, Artificial Sequence
  LFR1 of CD20-Fab-hole
QIVLSQSPAILSASPGEKVTMTC

SEQ ID NO: 33 - protein, 10 aa, Artificial Sequence
  LCDR1 of CD20-Fab-hole
RASSSVSYIH

SEQ ID NO: 34 - protein, 15 aa, Artificial Sequence
  LFR2 of CD20-Fab-hole
WFQQKPGSSPKPWIY

SEQ ID NO: 35 - protein, 7 aa, Artificial Sequence
  LCDR2 of CD20-Fab-hole
ATSNLAS

SEQ ID NO: 36 - protein, 32 aa, Artificial Sequence; identical to SEQ ID NO: 19
  LFR3 of CD20-Fab-hole

SEQ ID NO: 37 - protein, 9 aa, Artificial Sequence
  LCDR3 of CD20-Fab-hole
QQWTSNPPT

SEQ ID NO: 38 - protein, 10 aa, Artificial Sequence
  LFR4 of CD20-Fab-hole
FGGGTKLEIK

SEQ ID NO: 39 - protein, 107 aa, Artificial Sequence
  Ckappa of CD20-Fab-hole
RTAAAPSVFIFPPSDEQLKSGTASVVCLLNNFYPREAKVQWKVDNALQSGNSQESVTEQDSKDSTYSLSSTLTLSKADYEKHKVYACEVTHQGLSSPVTKSFNRGEC

SEQ ID NO: 40 - protein, 40 aa, Artificial Sequence
  Linker of CD20-Fab-hole
GGGGSGGGGSGGGGSGSGGSGGGGSGGGGSGGGGSGSGSS

SEQ ID NO: 41 - protein, 30 aa, Artificial Sequence; identical to SEQ ID NO: 23
  HFR1 of CD20-Fab-hole

SEQ ID NO: 42 - protein, 5 aa, Artificial Sequence
  HCDR1 of CD20-Fab-hole
SYNMH

SEQ ID NO: 43 - protein, 14 aa, Artificial Sequence
  HFR2 of CD20-Fab-hole
WVKQTPGRGLEWIG

SEQ ID NO: 44 - protein, 17 aa, Artificial Sequence
  HCDR2 of CD20-Fab-hole
AIYPGNGDTSYNQKFKG

SEQ ID NO: 45 - protein, 32 aa, Artificial Sequence; identical to SEQ ID NO: 27
  HFR3 of CD20-Fab-hole

SEQ ID NO: 46 - protein, 12 aa, Artificial Sequence
  HCDR3 of CD20-Fab-hole
STYYGGDWYFNV

SEQ ID NO: 47 - protein, 11 aa, Artificial Sequence
  HFR4 of CD20-Fab-hole
WGAGTTVTVSA

SEQ ID NO: 48 - protein, 103 aa, Artificial Sequence
  CH1 of CD20-Fab-hole
ASFKGPSVFPLAPSSKSTSGGTAALGCLVKDYFPEPVTVSWNSGALTSGVHTFPAVLQSSGLYSLSSVVTVPSSSLGTQTYICNVNHKPSNTKVDKKVEPKSC

SEQ ID NO: 49 - protein, 120 aa, Artificial Sequence; identical to SEQ ID NO: 30
  CH2 of CD20-Fab-hole

SEQ ID NO: 50 - protein, 107 aa, Artificial Sequence
  CH3 of CD20-Fab-hole
GQPREPQVYTLPPSRDELTKNQVSLSCAVKGFYPSDIAVEWESNGQPENNYKTTPPVLDSDGSFFLVSKLTVDKSRWQQGNVFSCSVMHEALHNHYTQKSLSLSPGK

SEQ ID NO: 51 - protein, 106 aa, Artificial Sequence [sequence omitted]

SEQ ID NO: 52 - protein, 121 aa, Artificial Sequence [sequence omitted]

SEQ ID NO: 53 - protein, 106 aa, Artificial Sequence [sequence omitted]

SEQ ID NO: 54 - protein, 121 aa, Artificial Sequence [sequence omitted]